European Patent Specification EP 3 903 829 B1, published May 3, 2023. Title: IMMUNOCONJUGATES WITH AN INTRACELLULARLY-CLEAVABLE LINKAGE. Applicant: IMMUNOMEDICS, INC. Application PCT/US09/66371. The sequence listing filed with the application follows.

SEQUENCE LISTING (15 sequences)

SEQ ID NO: 1 - protein, 44 aa, Homo sapiens
SHIQIPPGLTELLQGYTVEVLRQQPPDLVEFAVEYFTRLREARA

SEQ ID NO: 2 - protein, 45 aa, Homo sapiens
CGHIQIPPGLTELLQGYTVEVLRQQPPDLVEFAVEYFTRLREARA

SEQ ID NO: 3 - protein, 17 aa, Homo sapiens
QIEYLAKQIVDNAIQQA

SEQ ID NO: 4 - protein, 21 aa, Homo sapiens
CGQIEYLAKQIVDNAIQQAGC

SEQ ID NO: 5 - protein, 17 aa, Artificial Sequence
  Description of Artificial Sequence: Synthetic peptide
QIEYVAKQIVDYAIHQA

SEQ ID NO: 6 - protein, 17 aa, Artificial Sequence
  Description of Artificial Sequence: Synthetic peptide
QIEYKAKQIVDHAIHQA

SEQ ID NO: 7 - protein, 17 aa, Artificial Sequence
  Description of Artificial Sequence: Synthetic peptide
QIEYHAKQIVDHAIHQA

SEQ ID NO: 8 - protein, 17 aa, Artificial Sequence
  Description of Artificial Sequence: Synthetic peptide
QIEYVAKQIVDHAIHQA

SEQ ID NO: 9 - protein, 24 aa, Artificial Sequence
  Description of Artificial Sequence: Synthetic peptide
DLIEEAASRIVDAVIEQVKAAGAY

SEQ ID NO: 10 - protein, 18 aa, Artificial Sequence
  Description of Artificial Sequence: Synthetic peptide
LEQYANQLADQIIKEATE

SEQ ID NO: 11 - protein, 20 aa, Artificial Sequence
  Description of Artificial Sequence: Synthetic peptide
FEELAWKIAKMIWSDVFQQC

SEQ ID NO: 12 - protein, 25 aa, Homo sapiens
PEDAELVRLSKRLVENAVLKAVQQY

SEQ ID NO: 13 - protein, 25 aa, Homo sapiens
PEDAELVRTSKRLVENAVLKAVQQY

SEQ ID NO: 14 - protein, 25 aa, Homo sapiens
PEDAELVRLSKRDVENAVLKAVQQY

SEQ ID NO: 15 - protein, 4 aa, Artificial Sequence
  Description of Artificial Sequence: Synthetic peptide
ALAL